European Patent Application EP 4 431 612 A1, published September 18, 2024. Title: Verfahren zur Herstellung von Corytuberin und Salutaridin. Applicant: Universitaet Graz. Application EP. The sequence listing filed with the application follows.

SEQUENCE LISTING (30 sequences)

SEQ ID NO: 1 - protein, 343 aa, Papaver somniferum
  REGION 1..343: note = N-terminaler Histidin-tag; Mittels Sequenzierung bestimmte Aminosaeuresequenz
MAHHHHHHSAALEVLFQGPGYQMESSGVPVITLGSGKVMPVLGMGTFEKVGKGSERERLAILKAIEVGYRYFDTAAAYETEEVLGEAIAEALQLGLVKSRDELFISSMLWCTDAHADRVLLALQNSLRNLKLEYVDLYMLPFPASLKPGKITMDIPEEDICRMDYRSVWAAMEECQNLGFTKSIGVSNFSCKKLQELMATANIPPAVNQVEMSPAFQQKKLREYCNANNILVSAISVLGSNGTPWGSNAVLGSEVLKKIAMAKGKSVAQVSMRWVYEQGASLVVKSFSEERLRENLNIFDWELTKEDHEKIGEIPQCRILSAYFLVSPNGPFKSQEELWDDEA

SEQ ID NO: 2 - DNA, 1029 bp, Papaver somniferum
  misc_feature 1..1029: note = N-terminaler Histidin-tag; Fuer Sequenz-ID Nr. 1 kodierende Sequenz
  source 1..1029: mol_type = genomic DNA
atggcacatcaccaccaccatcactccgcggctcttgaagtcctctttcagggacccgggtaccagatggagagtagtggtgtaccagtaatcactctgggctcgggcaaggtgatgcctgttctgggcatgggaacatttgagaaagttggtaaagggtccgaaagagagaggttggcgattttaaaagcgatagaggtgggttacagatacttcgatacagctgctgcatacgaaactgaagaggttcttggagaagctattgctgaagcacttcaacttggcctagtcaaatctcgagatgaacttttcatcagttccatgctctggtgcactgatgctcacgctgatcgtgtcctcctcgctcttcagaattcgctgaggaatcttaaattggagtatgtggatctatatatgttacccttcccggcaagcttgaagcctgggaagataacgatggacataccagaggaagatatttgtcgcatggactacaggtctgtatgggcagccatggaagagtgtcaaaaccttggcttcactaaatcaatcggtgttagcaatttctcctgcaaaaagcttcaggaattgatggcgaccgccaacatccctccagctgtgaatcaagtggagatgagcccggctttccaacaaaagaagctgagagagtattgcaacgcaaataatatattagtcagtgcaatctctgtactgggatcaaacggaaccccatggggctccaatgcagttttgggttctgaggtgcttaagaaaattgctatggccaaaggaaaatctgttgctcaggttagtatgagatgggtttacgagcaaggcgcgagtcttgtggtaaaaagtttcagtgaagagagattgagggaaaacttgaacatatttgactgggaactcactaaggaagaccatgaaaagatcggtgagattccacagtgcagaatcttgagtgcttattttttggtctcacctaatggacctttcaaatctcaagaagagttgtgggatgatgaagct

SEQ ID NO: 3 - protein, 325 aa, Streptomyces aurantiacus
  REGION 1..325: note = N-terminaler Histidin-tag; N-terminale thrombin recognition and cleavage site; Codon-optimiert fuer E. coli; Mittels Sequenzierung bestimmte Aminosaeuresequenz
MGSSHHHHHHSSGLVPRGSHMATTTNSTNPTTASTLTPVTVIGLGAMGQALAGAFLKAGHPTTIWNRSPGKGEDLVARGATRAATPAEAVRAGEVVVVCVVDYEASQSILEPIAADLAGRVLVNVTSDAPERAREAGEWAAEHDIAYLDGAVMIPTVMIGTPDALLFYSGDKAAYDKHEGLLKSLGGQSAYVGADHGLAAVYDLSMLDFMFTSMSGLVHGYALAAKDGVPAASIAPFLKSHISLLSLLVEETAKNLDEGAYPGAEANLAMEVEGIEHILHAAERRGLDVSVLRGVRDVAQRAVDLGHGADSWSATVEGARNPAKL

SEQ ID NO: 4 - DNA, 975 bp, Streptomyces aurantiacus
  misc_feature 1..975: note = N-terminaler Histidin-tag; N-terminale thrombin recognition and cleavage site; Codon-optimiert fuer E. coli; Fuer Sequenz-ID Nr. 3 kodierende Sequenz
  source 1..975: mol_type = genomic DNA
atgggcagcagccatcatcatcatcatcacagcagcggcctggtgccgcgcggcagccatatggcaaccaccaccaatagtaccaatccgaccaccgcaagtaccctgaccccggtgaccgttattggtctgggtgccatgggccaggccctggcaggtgcatttctgaaagcaggtcatccgaccaccatttggaatcgtagcccgggtaaaggtgaagatctggtggcacgtggtgcaacccgcgccgcaacccctgcagaagcagtgcgtgcaggcgaagttgtggttgtgtgcgttgttgattatgaagccagccagagcattctggaaccgattgcagccgatctggcaggccgcgtgctggtgaatgtgaccagtgatgcaccggaacgcgcccgtgaagcaggtgaatgggccgccgaacatgatattgcctatctggatggtgcagttatgattccgaccgtgatgattggtaccccggatgcactgctgttttatagcggtgacaaagccgcatacgataaacatgaaggcctgctgaaaagcctgggtggccagagcgcatacgttggcgccgatcatggcctggccgcagtgtatgatctgagcatgctggattttatgtttaccagcatgagtggtctggttcatggctatgccctggccgccaaagatggcgtgccggcagccagtattgcaccgtttctgaaaagtcatattagcctgctgagcctgctggtggaagaaaccgccaaaaatctggatgaaggcgcatatccgggcgcagaagccaatctggcaatggaagtggaaggtattgaacatattctgcatgccgccgaacgccgtggtctggatgttagtgtgctgcgtggtgtgcgcgatgttgcccagcgcgccgtggatctgggtcatggtgccgatagttggagcgcaaccgttgaaggtgcacgcaatccggccaagctt

SEQ ID NO: 5 - protein, 737 aa, Arabidopsis thaliana
  REGION 1..737: note = N-terminales Flanking MG ; C-terminaler S-tag; Codon-optimiert fuer E. coli; Mittels Sequenzierung bestimmte Aminosaeuresequenz
MGMSSSSSSSTSMIDLMAAIIKGEPVIVSDPANASAYESVAAELSSMLIENRQFAMIVTTSIAVLIGCIVMLVWRRSGSGNSKRVEPLKPLVIKPREEEIDDGRKKVTIFFGTQTGTAEGFAKALGEEAKARYEKTRFKIVDLDDYAADDDEYEEKLKKEDVAFFFLATYGDGEPTDNAARFYKWFTEGNDRGEWLKNLKYGVFGLGNRQYEHFNKVAKVVDDILVEQGAQRLVQVGLGDDDQCIEDDFTAWREALWPELDTILREEGDTAVATPYTAAVLEYRVSIHDSEDAKFNDINMANGNGYTVFDAQHPYKANVAVKRELHTPESDRSCIHLEFDIAGSGLTYETGDHVGVLCDNLSETVDEALRLLDMSPDTYFSLHAEKEDGTPISSSLPPPFPPCNLRTALTRYACLLSSPKKSALVALAAHASDPTEAERLKHLASPAGKDEYSKWVVESQRSLLEVMAEFPSAKPPLGVFFAGVAPRLQPRFYSISSSPKIAETRIHVTCALVYEKMPTGRIHKGVCSTWMKNAVPYEKSENCSSAPIFVRQSNFKLPSDSKVPIIMIGPGTGLAPFRGFLQERLALVESGVELGPSVLFFGCRNRRMDFIYEEELQRFVESGALAELSVAFSREGPTKEYVQHKMMDKASDIWNMISQGAYLYVCGDAKGMARDVHRSLHTIAQEQGSMDSTKAEGFVKNLQTSGRYLRDVWLESGKETAAAKFERQHMDSSTSAA

SEQ ID NO: 6 - DNA, 2211 bp, Arabidopsis thaliana
  misc_feature 1..2211: note = N-terminales Flanking MG ; C-terminaler S-tag; Codon-optimiert fuer E. coli; Fuer Sequenz-ID Nr. 5 kodierende Sequenz
  source 1..2211: mol_type = genomic DNA
atgggaatgagtagcagcagtagtagtagtaccagcatgattgatctgatggccgcaattattaagggtgaaccggttattgtgagcgatccggccaatgccagtgcctatgaaagtgtggccgcagaactgagtagcatgctgattgaaaatcgccagtttgcaatgattgtgaccaccagtattgcagtgctgattggctgtattgttatgctggtttggcgtcgtagtggtagcggcaatagtaaacgtgttgaaccgctgaaaccgctggttattaagccgcgcgaagaagaaattgatgatggtcgcaaaaaagtgaccattttctttggtacccagaccggcaccgccgaaggctttgcaaaagcactgggtgaagaagcaaaagcacgttatgaaaaaacccgctttaaaattgtggatctggatgattatgcagccgatgatgatgaatatgaagaaaaactgaagaaggaagatgtggcctttttctttctggccacctatggtgacggtgaaccgaccgataatgccgcccgcttttataaatggtttaccgaaggtaatgaccgtggtgaatggctgaaaaatctgaaatatggtgtgtttggtctgggtaatcgccagtatgaacattttaataaggtggcaaaagtggttgatgatattctggtggaacagggcgcccagcgcctggttcaggttggcctgggcgatgatgatcagtgcattgaagatgattttaccgcctggcgcgaagcactgtggccggaactggataccattctgcgcgaagaaggtgacaccgcagtggcaaccccgtataccgcagccgttctggaatatcgtgtgagcattcatgatagtgaagatgccaaattcaatgatattaacatggcaaatggcaatggttataccgtttttgatgcacagcatccgtataaagccaatgtggccgttaaacgtgaactgcataccccggaaagtgatcgtagctgcattcatctggaatttgatattgcaggtagtggcctgacctatgaaaccggtgaccatgtgggtgttctgtgtgataatctgagtgaaaccgtggatgaagcactgcgcctgctggatatgagcccggatacctattttagcctgcatgccgaaaaagaagatggcaccccgattagcagtagtctgccgccgccgtttccgccgtgcaatctgcgcaccgcactgacccgttatgcatgcctgctgagcagcccgaaaaaatcagccctggtggccctggcagcccatgcctcagatccgaccgaagccgaacgcctgaaacatctggcaagtccggccggcaaagatgaatatagcaaatgggtggttgaaagccagcgcagcctgctggaagtgatggccgaatttccgagcgcaaaaccgccgctgggcgttttctttgcaggcgttgccccgcgtctgcagccgagattttatagcattagtagcagcccgaagattgcagaaacccgcattcatgtgacctgtgcactggtgtatgaaaaaatgccgaccggtcgtattcataaaggtgtttgtagtacctggatgaaaaatgcagtgccgtatgaaaaaagcgaaaattgtagcagcgcaccgatttttgtgcgccagagcaattttaaactgccgagcgatagcaaagttccgattattatgattggtccgggtaccggtctggcaccgtttcgtggctttctgcaggaacgcctggccctggtggaaagtggtgtggaactgggcccgagtgtgctgtttttcggctgccgcaatcgccgtatggattttatctatgaagaagaactgcagcgctttgttgaaagcggtgccctggccgaactgagtgttgcctttagtcgcgaaggtccgaccaaagaatatgttcagcataaaatgatggacaaagccagtgatatttggaatatgattagccagggtgcctatctgtatgtttgcggcgatgccaaaggtatggcacgtgatgtgcatcgcagtctgcataccattgcacaggaacagggcagcatggatagtaccaaagccgaaggttttgtgaaaaatctgcagaccagtggccgctatctgcgcgatgtgtggctcgagtctggtaaagaaaccgctgctgcgaaatttgaacgccagcacatggactcgtctactagcgcagct

SEQ ID NO: 7 - protein, 515 aa, Papaver somniferum
  REGION 1..515: note = N-terminales Flanking MG ; C-terminaler His-tag; Codon-optimiert fuer E. coli; Mittels Sequenzierung bestimmte Aminosaeuresequenz
MGMAPINIEGNDFWMIACTVIIVFALVKFMFSKISFYQSANTTEWPAGPKTLPIIGNLHQLGGGVPLQVALANLAKVYGGAFTIWIGSWVPMIVISDIDNAREVLVNKSADYSARDVPDILKIITANGKNIADCDSGPFWHNLKKGLQSCINPSNVMSLSRLQEKDMQNLIKSMQERASQHNGIIKPLDHAKEASMRLLSRVIFGHDFSNEDLVIGVKDALDEMVRISGLASLADAFKIAKYLPSQRKNIRDMYATRDRVYNLIQPHIVPNLPENSFLHFLTSQDYSDEIIYSMVLEIFGLGVDSTAATAVWALSFLVGEQEIQEKLYREINNRTGGQRPVKVVDLKELPYLQAVMKETLRMKPIAPLAVPHVAAKDTTFKGRRIVKGTKVMVNLYAIHHDPNVFPAPYKFMPERFLKDVNSDGRFGDINTMESSLIPFGAGMRICGGVELAKQMVAFALASMVNEFKWDCVSEGKLPDLSEAISFILYMKNPLEAKITPRTKPFRQLEHHHHHH

SEQ ID NO: 8 - DNA, 1545 bp, Papaver somniferum
  misc_feature 1..1545: note = N-terminales Flanking MG ; C-terminaler His-tag; Codon-optimiert fuer E. coli; Fuer Sequenz-ID Nr. 7 kodierende Sequenz
  source 1..1545: mol_type = genomic DNA
atgggaatggcccctattaatattgaaggtaatgatttttggatgatcgcatgcaccgtgattattgtgtttgcactggttaaattcatgtttagtaagattagcttctaccagagtgcaaataccaccgaatggccggccggtccgaaaaccctgccgattattggcaatctgcatcagctgggcggtggcgtgccgctgcaggttgctctggccaatctggcaaaagtttatggcggcgcctttaccatttggattggtagttgggttccgatgattgttattagtgatattgataacgcgcgtgaagtgctggttaataagagcgcagattatagtgcccgtgatgtgccggatattctgaaaattattaccgccaatggcaaaaatatcgcagattgcgatagcggtccgttttggcataatctgaaaaaaggcctgcagagctgcattaatccgagtaatgtgatgagcctgagtcgcctgcaggaaaaagatatgcagaatctgattaagagtatgcaggaacgtgcaagtcagcataatggtattattaagccgctggatcatgcaaaagaagcaagcatgcgcctgctgagtcgcgtgatttttggtcatgattttagtaatgaggacctggttattggtgttaaagatgcactggatgaaatggttcgtattagtggcctggccagcctggccgatgcctttaaaattgcaaaatatctgccgagtcagcgcaaaaatattcgcgatatgtatgccacccgtgatcgtgtttataatctgattcagccgcatattgttccgaatctgccggaaaatagctttctgcattttctgaccagccaggattatagcgatgaaattatctatagtatggtgctggaaattttcggtctgggcgtggatagtaccgcagcaaccgcagtgtgggccctgagttttctggttggcgaacaggaaattcaggaaaaactgtatcgtgaaattaacaatcgtaccggtggtcagcgcccggttaaagttgttgatctgaaagaactgccgtatctgcaggccgttatgaaagaaaccctgcgcatgaaaccgattgcaccgctggccgttccgcatgtggccgcaaaagataccacctttaaaggccgtcgcattgttaaaggcaccaaagttatggtgaatctgtatgcaattcatcatgatccgaatgtgtttccggcaccgtataaattcatgccggaacgttttctgaaagatgttaatagtgatggtcgttttggtgacattaatacaatggaaagcagcctgattccgtttggtgcaggtatgcgcatttgtggcggtgttgaactggccaaacagatggtggcatttgccctggcaagcatggttaatgaattcaaatgggattgcgttagcgaaggtaaactgccggatctgagtgaagccattagctttattctgtatatgaaaaacccgctggaagcaaaaattaccccgcgtaccaaaccgtttcgccagctcgagcaccaccaccaccaccac

SEQ ID NO: 9 - protein, 486 aa, Papaver somniferum
  REGION 1..486: note = N-terminales Entfernen der Transmembrandomaene (29 Aminosaeuren) und N-terminales Flanking MG ; C-terminaler His-tag; Codon-optimiert fuer E. coli; Mittels Sequenzierung bestimmte Aminosaeuresequenz
MGMKISFYQSANTTEWPAGPKTLPIIGNLHQLGGGVPLQVALANLAKVYGGAFTIWIGSWVPMIVISDIDNAREVLVNKSADYSARDVPDILKIITANGKNIADCDSGPFWHNLKKGLQSCINPSNVMSLSRLQEKDMQNLIKSMQERASQHNGIIKPLDHAKEASMRLLSRVIFGHDFSNEDLVIGVKDALDEMVRISGLASLADAFKIAKYLPSQRKNIRDMYATRDRVYNLIQPHIVPNLPENSFLHFLTSQDYSDEIIYSMVLEIFGLGVDSTAATAVWALSFLVGEQEIQEKLYREINNRTGGQRPVKVVDLKELPYLQAVMKETLRMKPIAPLAVPHVAAKDTTFKGRRIVKGTKVMVNLYAIHHDPNVFPAPYKFMPERFLKDVNSDGRFGDINTMESSLIPFGAGMRICGGVELAKQMVAFALASMVNEFKWDCVSEGKLPDLSEAISFILYMKNPLEAKITPRTKPFRQLEHHHHHH

SEQ ID NO: 10 - DNA, 1458 bp, Papaver somniferum
  misc_feature 1..1458: note = N-terminales Entfernen der Transmembrandomaene (29 Aminosaeuren) und N-terminales Flanking MG ; C-terminaler His-tag; Codon-optimiert fuer E. coli; Fuer Sequenz-ID Nr. 9 kodierende Sequenz
  source 1..1458: mol_type = genomic DNA
atgggaatgaagatcagtttctaccagagcgcaaataccaccgaatggccggccggtccgaaaaccctgccgattattggtaatctgcatcagctgggcggcggcgttccgctgcaggttgctctggcaaatctggccaaagtttatggcggtgcctttaccatttggattggtagctgggttccgatgattgttattagtgatattgataacgcccgtgaagttctggttaataagagcgcagattatagcgcacgcgatgtgccggatattctgaaaattattaccgccaatggtaaaaatatcgccgattgcgatagcggcccgttttggcataatctgaaaaaaggcctgcagagctgcattaatccgagtaatgttatgagcctgagtcgcctgcaggaaaaagatatgcagaatctgattaagagcatgcaggaacgcgcaagccagcataatggcattattaagccgctggatcatgcaaaagaagcaagcatgcgtctgctgagtcgtgtgatttttggccatgattttagcaatgaagatctggttattggcgtgaaagatgccctggatgaaatggttcgtattagcggcctggcaagcctggcagatgcattcaaaattgccaaatatctgccgagtcagcgcaaaaatattcgtgatatgtatgccacccgtgatcgtgtgtataatctgattcagccgcatattgttccgaatctgccggaaaatagttttctgcattttctgaccagccaggattatagtgatgaaattatctatagcatggtgctggaaatttttggtctgggtgttgatagtaccgcagcaaccgcagtgtgggccctgagttttctggtgggcgaacaggaaattcaggaaaaactgtatcgcgaaattaataatcgcaccggtggtcagcgtccggttaaagttgtggatctgaaagaactgccgtatctgcaggcagtgatgaaagaaaccctgcgcatgaaaccgattgcaccgctggccgttccgcatgtggccgcaaaagataccacctttaaaggtcgccgcattgttaaaggcaccaaagtgatggttaatctgtatgccattcatcatgatccgaatgtttttccggcaccgtataaattcatgccggaacgttttctgaaagatgtgaatagcgatggccgctttggcgatattaatacaatggaaagcagcctgattccgtttggtgccggtatgcgtatttgtggcggtgtggaactggcaaaacagatggttgcatttgcactggccagtatggttaatgaattcaaatgggattgtgtgagcgaaggcaaactgccggatctgagtgaagccattagctttattctgtatatgaaaaacccgctggaagccaaaattaccccgcgcaccaaaccgtttcgtcagctcgagcaccaccaccaccaccac

SEQ ID NO: 11 - protein, 504 aa, Papaver somniferum
  REGION 1..504: note = N-terminales Flanking MG ; C-terminaler His-tag, Codon-optimiert fuer E. coli; Mittels Sequenzierung bestimmte Aminosaeuresequenz
MGMEESLWVVTATVVVVFAIAKLLKKSSSISTMEWPKGPKKLPIIGNLHQLGGEAFHVVLANLAKIHGTVMTIWVGAWRPMIVISDIDNAREVLVNKSADYSARDVPDILKIITANGKNIADCDSGPFWHNLKKGLQSCINPSNVMSLSRLQEKDMQNLIKSMQERASQHNGIIKPLDHAKEASMRLLSRVIFGHDFSNEDLVIGVKDALDEMVRISGLASLADAFKIAKYLPSQRKNIRDMYATRDRVYNLIQPHIVPNLPANSFLYFLTSQDYSDEIIYSMVLEIFGLGVDSTAATAVWALSFLVGEQEIQEKLYREINNRTGGQRPVKVVDLKELPYLQAVMKETLRMKPIAPLAVPHVAAKDTTFKGRRIVKGTKVMVNLYAIHHDPNVFPAPYKFMPERFLKDVNSDGRFGDINTMESSLIPFGAGMRICGGVELAKQMVAFALASMVNEFKWDCVSEGKLPDLSEAISFILYMKNPLEAKITPRTKPFRQLEHHHHHH

SEQ ID NO: 12 - DNA, 1512 bp, Papaver somniferum
  misc_feature 1..1512: note = N-terminales Flanking MG ; C-terminaler His-tag, Codon-optimiert fuer E. coli; Fuer Sequenz-ID Nr. 11 kodierende Sequenz
  source 1..1512: mol_type = genomic DNA
atgggaatggaagaaagtctgtgggttgttaccgccaccgtggttgtggtttttgccattgcaaaactgctgaaaaaatctagcagtattagcacaatggaatggccgaaaggcccgaaaaaactgccgattattggcaatctgcatcagctgggcggtgaagcctttcatgtggttctggccaatctggcaaaaattcatggcaccgttatgaccatttgggtgggtgcctggcgtccgatgattgtgattagcgatattgataatgcccgtgaagtgctggttaataagagcgcagattatagcgcccgcgatgttccggatattctgaaaattattaccgcaaatggtaaaaacatcgccgattgtgatagcggcccgttttggcataatctgaaaaaaggtctgcagagttgcattaatccgagtaatgtgatgagcctgagtcgtctgcaggaaaaagatatgcagaatctgattaagagcatgcaggaacgtgcaagccagcataatggcattattaagccgctggatcatgccaaagaagccagtatgcgtctgctgagccgtgtgatttttggccatgattttagcaatgaagatctggttattggcgttaaagatgccctggatgaaatggttcgcattagcggtctggccagcctggcagatgcattcaaaattgcaaaatatctgccgagccagcgcaaaaatattcgcgatatgtatgccacccgcgatcgtgtgtataatctgattcagccgcatattgttccgaatctgccggccaatagttttctgtattttctgaccagtcaggattatagcgatgaaattatctatagtatggtgctggaaattttcggcctgggtgtggatagcaccgcagcaaccgcagtttgggccctgagttttctggtgggtgaacaggaaattcaggaaaaactgtatcgcgaaattaataatcgtaccggtggtcagcgtccggttaaagtggtggatctgaaagaactgccgtatctgcaggcagtgatgaaagaaaccctgcgcatgaaaccgattgccccgctggccgtgccgcatgttgcagcaaaagataccacctttaaaggtcgccgcattgttaaaggtaccaaagtgatggttaatctgtatgcaattcatcatgatccgaatgtttttccggcaccgtataaattcatgccggaacgctttctgaaagatgttaatagcgatggccgctttggtgacattaatacaatggaaagcagcctgattccgtttggtgccggtatgcgcatttgcggcggcgtggaactggcaaaacagatggttgcctttgccctggccagtatggtgaatgaattcaaatgggattgtgtgagtgaaggcaaactgccggatctgagcgaagcaattagctttattctgtatatgaagaacccgctggaagcaaaaattaccccgcgcaccaaaccgtttcgccagctcgagcaccaccaccaccaccac

SEQ ID NO: 13 - protein, 771 aa, Papaver somniferum
  REGION 1..771: note = N-terminaler His-tag; N-terminaler GST-tag; Codon-optimiert fuer E. coli; Mittels Sequenzierung bestimmte Aminosaeuresequenz
MGSSHHHHHHGTSPILGYWKIKGLVQPTRLLLEYLEEKYEEHLYERDEGDKWRNKKFELGLEFPNLPYYIDGDVKLTQSMAIIRYIADKHNMLGGCPKERAEISMLEGAVLDIRYGVSRIAYSKDFETLKVDFLSKLPEMLKMFEDRLCHKTYLNGDHVTHPDFMLYDALDVVLYMDPMCLDAFPKLVCFKKRIEAIPQIDKYLKSSKYIAWPLQGWQATFGGGDHPPKSDGTDYDIPTTENLYFQGHMASMTGGQQMGRGSEFELMAPINIEGNDFWMIACTVIIVFALVKFMFSKISFYQSANTTEWPAGPKTLPIIGNLHQLGGGVPLQVALANLAKVYGGAFTIWIGSWVPMIVISDIDNAREVLVNKSADYSARDVPDILKIITANGKNIADCDSGPFWHNLKKGLQSCINPSNVMSLSRLQEKDMQNLIKSMQERASQHNGIIKPLDHAKEASMRLLSRVIFGHDFSNEDLVIGVKDALDEMVRISGLASLADAFKIAKYLPSQRKNIRDMYATRDRVYNLIQPHIVPNLPENSFLHFLTSQDYSDEIIYSMVLEIFGLGVDSTAATAVWALSFLVGEQEIQEKLYREINNRTGGQRPVKVVDLKELPYLQAVMKETLRMKPIAPLAVPHVAAKDTTFKGRRIVKGTKVMVNLYAIHHDPNVFPAPYKFMPERFLKDVNSDGRFGDINTMESSLIPFGAGMRICGGVELAKQMVAFALASMVNEFKWDCVSEGKLPDLSEAISFILYMKNPLEAKITPRTKPFRQ

SEQ ID NO: 14 - DNA, 2313 bp, Papaver somniferum
  misc_feature 1..2313: note = N-terminaler His-tag; N-terminaler GST-tag; Codon-optimiert fuer E. coli; Fuer Sequenz-ID Nr. 13 kodierende Sequenz
  source 1..2313: mol_type = genomic DNA
atgggcagcagccatcatcatcatcatcacggtacctcccctatactaggttattggaaaattaagggccttgtgcaacccactcgacttcttttggaatatcttgaagaaaaatatgaagagcatttgtatgagcgcgatgaaggtgataaatggcgaaacaaaaagtttgaattgggtttggagtttcccaatcttccttattatattgatggtgatgttaaattaacacagtctatggccatcatacgttatatagctgacaagcacaacatgttgggtggttgtccaaaagagcgtgcagagatttcaatgcttgaaggagcggttttggatattagatacggtgtttcgagaattgcatatagtaaagactttgaaactctcaaagttgattttcttagcaagctacctgaaatgctgaaaatgttcgaagatcgtttatgtcataaaacatatttaaatggtgatcatgtaacccatcctgacttcatgttgtatgacgctcttgatgttgttttatacatggacccaatgtgcctggatgcgttcccaaaattagtttgttttaaaaaacgtattgaagctatcccacaaattgataagtacttgaaatccagcaagtatatagcatggcctttgcagggctggcaagccacgtttggtggtggcgaccatcctccaaaatcggatggtaccgattacgatatcccaacgaccgaaaacctttacttccagggccatatggctagcatgactggtggacagcaaatgggtcgcggatccgaattcgagctcatggcccctattaatattgaaggtaatgatttttggatgatcgcatgcaccgtgattattgtgtttgcactggttaaattcatgtttagtaagattagcttctaccagagtgcaaataccaccgaatggccggccggtccgaaaaccctgccgattattggcaatctgcatcagctgggcggtggcgtgccgctgcaggttgctctggccaatctggcaaaagtttatggcggcgcctttaccatttggattggtagttgggttccgatgattgttattagtgatattgataacgcgcgtgaagtgctggttaataagagcgcagattatagtgcccgtgatgtgccggatattctgaaaattattaccgccaatggcaaaaatatcgcagattgcgatagcggtccgttttggcataatctgaaaaaaggcctgcagagctgcattaatccgagtaatgtgatgagcctgagtcgcctgcaggaaaaagatatgcagaatctgattaagagtatgcaggaacgtgcaagtcagcataatggtattattaagccgctggatcatgcaaaagaagcaagcatgcgcctgctgagtcgcgtgatttttggtcatgattttagtaatgaggacctggttattggtgttaaagatgcactggatgaaatggttcgtattagtggcctggccagcctggccgatgcctttaaaattgcaaaatatctgccgagtcagcgcaaaaatattcgcgatatgtatgccacccgtgatcgtgtttataatctgattcagccgcatattgttccgaatctgccggaaaatagctttctgcattttctgaccagccaggattatagcgatgaaattatctatagtatggtgctggaaattttcggtctgggcgtggatagtaccgcagcaaccgcagtgtgggccctgagttttctggttggcgaacaggaaattcaggaaaaactgtatcgtgaaattaacaatcgtaccggtggtcagcgcccggttaaagttgttgatctgaaagaactgccgtatctgcaggccgttatgaaagaaaccctgcgcatgaaaccgattgcaccgctggccgttccgcatgtggccgcaaaagataccacctttaaaggccgtcgcattgttaaaggcaccaaagttatggtgaatctgtatgcaattcatcatgatccgaatgtgtttccggcaccgtataaattcatgccggaacgttttctgaaagatgttaatagtgatggtcgttttggtgacattaatacaatggaaagcagcctgattccgtttggtgcaggtatgcgcatttgtggcggtgttgaactggccaaacagatggtggcatttgccctggcaagcatggttaatgaattcaaatgggattgcgttagcgaaggtaaactgccggatctgagtgaagccattagctttattctgtatatgaaaaacccgctggaagcaaaaattaccccgcgtaccaaaccgtttcgccag

SEQ ID NO: 15 - protein, 742 aa, Papaver somniferum
  REGION 1..742: note = N-terminales Entfernen der Transmembrandomaene (29 Aminosaeuren); N-terminaler His-tag; N-terminaler GST-tag; Codon-optimiert fuer E. coli; Mittels Sequenzierung bestimmte Aminosaeuresequenz
MGSSHHHHHHGTSPILGYWKIKGLVQPTRLLLEYLEEKYEEHLYERDEGDKWRNKKFELGLEFPNLPYYIDGDVKLTQSMAIIRYIADKHNMLGGCPKERAEISMLEGAVLDIRYGVSRIAYSKDFETLKVDFLSKLPEMLKMFEDRLCHKTYLNGDHVTHPDFMLYDALDVVLYMDPMCLDAFPKLVCFKKRIEAIPQIDKYLKSSKYIAWPLQGWQATFGGGDHPPKSDGTDYDIPTTENLYFQGHMASMTGGQQMGRGSEFELMKISFYQSANTTEWPAGPKTLPIIGNLHQLGGGVPLQVALANLAKVYGGAFTIWIGSWVPMIVISDIDNAREVLVNKSADYSARDVPDILKIITANGKNIADCDSGPFWHNLKKGLQSCINPSNVMSLSRLQEKDMQNLIKSMQERASQHNGIIKPLDHAKEASMRLLSRVIFGHDFSNEDLVIGVKDALDEMVRISGLASLADAFKIAKYLPSQRKNIRDMYATRDRVYNLIQPHIVPNLPENSFLHFLTSQDYSDEIIYSMVLEIFGLGVDSTAATAVWALSFLVGEQEIQEKLYREINNRTGGQRPVKVVDLKELPYLQAVMKETLRMKPIAPLAVPHVAAKDTTFKGRRIVKGTKVMVNLYAIHHDPNVFPAPYKFMPERFLKDVNSDGRFGDINTMESSLIPFGAGMRICGGVELAKQMVAFALASMVNEFKWDCVSEGKLPDLSEAISFILYMKNPLEAKITPRTKPFRQ

SEQ ID NO: 16 - DNA, 2226 bp, Papaver somniferum
  misc_feature 1..2226: note = N-terminales Entfernen der Transmembrandomaene (29 Aminosaeuren); N-terminaler His-tag; N-terminaler GST-tag; Codon-optimiert fuer E. coli; Fuer Sequenz-ID Nr. 15 kodierende Sequenz
  source 1..2226: mol_type = genomic DNA
atgggcagcagccatcatcatcatcatcacggtacctcccctatactaggttattggaaaattaagggccttgtgcaacccactcgacttcttttggaatatcttgaagaaaaatatgaagagcatttgtatgagcgcgatgaaggtgataaatggcgaaacaaaaagtttgaattgggtttggagtttcccaatcttccttattatattgatggtgatgttaaattaacacagtctatggccatcatacgttatatagctgacaagcacaacatgttgggtggttgtccaaaagagcgtgcagagatttcaatgcttgaaggagcggttttggatattagatacggtgtttcgagaattgcatatagtaaagactttgaaactctcaaagttgattttcttagcaagctacctgaaatgctgaaaatgttcgaagatcgtttatgtcataaaacatatttaaatggtgatcatgtaacccatcctgacttcatgttgtatgacgctcttgatgttgttttatacatggacccaatgtgcctggatgcgttcccaaaattagtttgttttaaaaaacgtattgaagctatcccacaaattgataagtacttgaaatccagcaagtatatagcatggcctttgcagggctggcaagccacgtttggtggtggcgaccatcctccaaaatcggatggtaccgattacgatatcccaacgaccgaaaacctttacttccagggccatatggctagcatgactggtggacagcaaatgggtcgcggatccgaattcgagctcatgaagatcagtttctaccagagcgcaaataccaccgaatggccggccggtccgaaaaccctgccgattattggtaatctgcatcagctgggcggcggcgttccgctgcaggttgctctggcaaatctggccaaagtttatggcggtgcctttaccatttggattggtagctgggttccgatgattgttattagtgatattgataacgcccgtgaagttctggttaataagagcgcagattatagcgcacgcgatgtgccggatattctgaaaattattaccgccaatggtaaaaatatcgccgattgcgatagcggcccgttttggcataatctgaaaaaaggcctgcagagctgcattaatccgagtaatgttatgagcctgagtcgcctgcaggaaaaagatatgcagaatctgattaagagcatgcaggaacgcgcaagccagcataatggcattattaagccgctggatcatgcaaaagaagcaagcatgcgtctgctgagtcgtgtgatttttggccatgattttagcaatgaagatctggttattggcgtgaaagatgccctggatgaaatggttcgtattagcggcctggcaagcctggcagatgcattcaaaattgccaaatatctgccgagtcagcgcaaaaatattcgtgatatgtatgccacccgtgatcgtgtgtataatctgattcagccgcatattgttccgaatctgccggaaaatagttttctgcattttctgaccagccaggattatagtgatgaaattatctatagcatggtgctggaaatttttggtctgggtgttgatagtaccgcagcaaccgcagtgtgggccctgagttttctggtgggcgaacaggaaattcaggaaaaactgtatcgcgaaattaataatcgcaccggtggtcagcgtccggttaaagttgtggatctgaaagaactgccgtatctgcaggcagtgatgaaagaaaccctgcgcatgaaaccgattgcaccgctggccgttccgcatgtggccgcaaaagataccacctttaaaggtcgccgcattgttaaaggcaccaaagtgatggttaatctgtatgccattcatcatgatccgaatgtttttccggcaccgtataaattcatgccggaacgttttctgaaagatgtgaatagcgatggccgctttggcgatattaatacaatggaaagcagcctgattccgtttggtgccggtatgcgtatttgtggcggtgtggaactggcaaaacagatggttgcatttgcactggccagtatggttaatgaattcaaatgggattgtgtgagcgaaggcaaactgccggatctgagtgaagccattagctttattctgtatatgaaaaacccgctggaagccaaaattaccccgcgcaccaaaccgtttcgtcag

SEQ ID NO: 17 - protein, 633 aa, Papaver somniferum
  REGION 1..633: note = N-terminaler His-tag; N-terminaler SUMO-tag; Codon-optimiert fuer E. coli; Mittels Sequenzierung bestimmte Aminosaeuresequenz
MGSSHHHHHHHHGSGLVPRGSASMSDSEVNQEAKPEVKPEVKPETHINLKVSDGSSEIFFKIKKTTPLRRLMEAFAKRQGKEMDSLRFLYDGIRIQADQTPEDLDMEDNDIIEAHREQIGGRGSEFELMAPINIEGNDFWMIACTVIIVFALVKFMFSKISFYQSANTTEWPAGPKTLPIIGNLHQLGGGVPLQVALANLAKVYGGAFTIWIGSWVPMIVISDIDNAREVLVNKSADYSARDVPDILKIITANGKNIADCDSGPFWHNLKKGLQSCINPSNVMSLSRLQEKDMQNLIKSMQERASQHNGIIKPLDHAKEASMRLLSRVIFGHDFSNEDLVIGVKDALDEMVRISGLASLADAFKIAKYLPSQRKNIRDMYATRDRVYNLIQPHIVPNLPENSFLHFLTSQDYSDEIIYSMVLEIFGLGVDSTAATAVWALSFLVGEQEIQEKLYREINNRTGGQRPVKVVDLKELPYLQAVMKETLRMKPIAPLAVPHVAAKDTTFKGRRIVKGTKVMVNLYAIHHDPNVFPAPYKFMPERFLKDVNSDGRFGDINTMESSLIPFGAGMRICGGVELAKQMVAFALASMVNEFKWDCVSEGKLPDLSEAISFILYMKNPLEAKITPRTKPFRQ

SEQ ID NO: 18 - DNA, 1899 bp, Papaver somniferum
  misc_feature 1..1899: note = N-terminaler His-tag; N-terminaler SUMO-tag; Codon-optimiert fuer E. coli; Fuer Sequenz-ID Nr. 17 kodierende Sequenz
  source 1..1899: mol_type = genomic DNA
atgggcagcagccatcaccatcatcatcatcatcacggcagcggcctggtgccgcgcggcagcgctagcatgtcggactcagaagtcaatcaagaagctaagccagaggtcaagccagaagtcaagcctgagactcacatcaatttaaaggtgtccgatggatcttcagagatcttcttcaagatcaaaaagaccactcctttaagaaggctgatggaagcgttcgctaaaagacagggtaaggaaatggactccttaagattcttgtacgacggtattagaatacaagctgatcagacccctgaagatttggacatggaggataacgatattattgaggctcacagagaacagattggtggtcgcggatccgaattcgagctcatggcccctattaatattgaaggtaatgatttttggatgatcgcatgcaccgtgattattgtgtttgcactggttaaattcatgtttagtaagattagcttctaccagagtgcaaataccaccgaatggccggccggtccgaaaaccctgccgattattggcaatctgcatcagctgggcggtggcgtgccgctgcaggttgctctggccaatctggcaaaagtttatggcggcgcctttaccatttggattggtagttgggttccgatgattgttattagtgatattgataacgcgcgtgaagtgctggttaataagagcgcagattatagtgcccgtgatgtgccggatattctgaaaattattaccgccaatggcaaaaatatcgcagattgcgatagcggtccgttttggcataatctgaaaaaaggcctgcagagctgcattaatccgagtaatgtgatgagcctgagtcgcctgcaggaaaaagatatgcagaatctgattaagagtatgcaggaacgtgcaagtcagcataatggtattattaagccgctggatcatgcaaaagaagcaagcatgcgcctgctgagtcgcgtgatttttggtcatgattttagtaatgaggacctggttattggtgttaaagatgcactggatgaaatggttcgtattagtggcctggccagcctggccgatgcctttaaaattgcaaaatatctgccgagtcagcgcaaaaatattcgcgatatgtatgccacccgtgatcgtgtttataatctgattcagccgcatattgttccgaatctgccggaaaatagctttctgcattttctgaccagccaggattatagcgatgaaattatctatagtatggtgctggaaattttcggtctgggcgtggatagtaccgcagcaaccgcagtgtgggccctgagttttctggttggcgaacaggaaattcaggaaaaactgtatcgtgaaattaacaatcgtaccggtggtcagcgcccggttaaagttgttgatctgaaagaactgccgtatctgcaggccgttatgaaagaaaccctgcgcatgaaaccgattgcaccgctggccgttccgcatgtggccgcaaaagataccacctttaaaggccgtcgcattgttaaaggcaccaaagttatggtgaatctgtatgcaattcatcatgatccgaatgtgtttccggcaccgtataaattcatgccggaacgttttctgaaagatgttaatagtgatggtcgttttggtgacattaatacaatggaaagcagcctgattccgtttggtgcaggtatgcgcatttgtggcggtgttgaactggccaaacagatggtggcatttgccctggcaagcatggttaatgaattcaaatgggattgcgttagcgaaggtaaactgccggatctgagtgaagccattagctttattctgtatatgaaaaacccgctggaagcaaaaattaccccgcgtaccaaaccgtttcgccag

SEQ ID NO: 19 - protein, 604 aa, Papaver somniferum
  REGION 1..604: note = N-terminales Entfernen der Transmembrandomaene (29 Aminosaeuren); N-terminaler His-tag; N-terminaler SUMO-tag; Codon-optimiert fuer E. coli; Mittels Sequenzierung bestimmte Aminosaeuresequenz
MGSSHHHHHHHHGSGLVPRGSASMSDSEVNQEAKPEVKPEVKPETHINLKVSDGSSEIFFKIKKTTPLRRLMEAFAKRQGKEMDSLRFLYDGIRIQADQTPEDLDMEDNDIIEAHREQIGGRGSEFELMKISFYQSANTTEWPAGPKTLPIIGNLHQLGGGVPLQVALANLAKVYGGAFTIWIGSWVPMIVISDIDNAREVLVNKSADYSARDVPDILKIITANGKNIADCDSGPFWHNLKKGLQSCINPSNVMSLSRLQEKDMQNLIKSMQERASQHNGIIKPLDHAKEASMRLLSRVIFGHDFSNEDLVIGVKDALDEMVRISGLASLADAFKIAKYLPSQRKNIRDMYATRDRVYNLIQPHIVPNLPENSFLHFLTSQDYSDEIIYSMVLEIFGLGVDSTAATAVWALSFLVGEQEIQEKLYREINNRTGGQRPVKVVDLKELPYLQAVMKETLRMKPIAPLAVPHVAAKDTTFKGRRIVKGTKVMVNLYAIHHDPNVFPAPYKFMPERFLKDVNSDGRFGDINTMESSLIPFGAGMRICGGVELAKQMVAFALASMVNEFKWDCVSEGKLPDLSEAISFILYMKNPLEAKITPRTKPFRQ

SEQ ID NO: 20 - DNA, 1812 bp, Papaver somniferum
  misc_feature 1..1812: note = N-terminales Entfernen der Transmembrandomaene (29 Aminosaeuren); N-terminaler His-tag; N-terminaler SUMO-tag; Codon-optimiert fuer E. coli; Fuer Sequenz-ID Nr. 19 kodierende Sequenz
  source 1..1812: mol_type = genomic DNA
atgggcagcagccatcaccatcatcatcatcatcacggcagcggcctggtgccgcgcggcagcgctagcatgtcggactcagaagtcaatcaagaagctaagccagaggtcaagccagaagtcaagcctgagactcacatcaatttaaaggtgtccgatggatcttcagagatcttcttcaagatcaaaaagaccactcctttaagaaggctgatggaagcgttcgctaaaagacagggtaaggaaatggactccttaagattcttgtacgacggtattagaatacaagctgatcagacccctgaagatttggacatggaggataacgatattattgaggctcacagagaacagattggtggtcgcggatccgaattcgagctcatgaagatcagtttctaccagagcgcaaataccaccgaatggccggccggtccgaaaaccctgccgattattggtaatctgcatcagctgggcggcggcgttccgctgcaggttgctctggcaaatctggccaaagtttatggcggtgcctttaccatttggattggtagctgggttccgatgattgttattagtgatattgataacgcccgtgaagttctggttaataagagcgcagattatagcgcacgcgatgtgccggatattctgaaaattattaccgccaatggtaaaaatatcgccgattgcgatagcggcccgttttggcataatctgaaaaaaggcctgcagagctgcattaatccgagtaatgttatgagcctgagtcgcctgcaggaaaaagatatgcagaatctgattaagagcatgcaggaacgcgcaagccagcataatggcattattaagccgctggatcatgcaaaagaagcaagcatgcgtctgctgagtcgtgtgatttttggccatgattttagcaatgaagatctggttattggcgtgaaagatgccctggatgaaatggttcgtattagcggcctggcaagcctggcagatgcattcaaaattgccaaatatctgccgagtcagcgcaaaaatattcgtgatatgtatgccacccgtgatcgtgtgtataatctgattcagccgcatattgttccgaatctgccggaaaatagttttctgcattttctgaccagccaggattatagtgatgaaattatctatagcatggtgctggaaatttttggtctgggtgttgatagtaccgcagcaaccgcagtgtgggccctgagttttctggtgggcgaacaggaaattcaggaaaaactgtatcgcgaaattaataatcgcaccggtggtcagcgtccggttaaagttgtggatctgaaagaactgccgtatctgcaggcagtgatgaaagaaaccctgcgcatgaaaccgattgcaccgctggccgttccgcatgtggccgcaaaagataccacctttaaaggtcgccgcattgttaaaggcaccaaagtgatggttaatctgtatgccattcatcatgatccgaatgtttttccggcaccgtataaattcatgccggaacgttttctgaaagatgtgaatagcgatggccgctttggcgatattaatacaatggaaagcagcctgattccgtttggtgccggtatgcgtatttgtggcggtgtggaactggcaaaacagatggttgcatttgcactggccagtatggttaatgaattcaaatgggattgtgtgagcgaaggcaaactgccggatctgagtgaagccattagctttattctgtatatgaaaaacccgctggaagccaaaattaccccgcgcaccaaaccgtttcgtcag

SEQ ID NO: 21 - protein, 494 aa, Papaver somniferum
  REGION 1..494: note = N-terminales Austauschen der Transmembrandomaene (29 Aminosaeuren) mit der Sequenz ALLLAVFL und N-terminales Flanking MG ; C-terminaler His-tag; Codon-optimiert fuer E. coli; Mittels Sequenzierung bestimmte Aminosaeuresequenz
MGMALLLAVFLKISFYQSANTTEWPAGPKTLPIIGNLHQLGGGVPLQVALANLAKVYGGAFTIWIGSWVPMIVISDIDNAREVLVNKSADYSARDVPDILKIITANGKNIADCDSGPFWHNLKKGLQSCINPSNVMSLSRLQEKDMQNLIKSMQERASQHNGIIKPLDHAKEASMRLLSRVIFGHDFSNEDLVIGVKDALDEMVRISGLASLADAFKIAKYLPSQRKNIRDMYATRDRVYNLIQPHIVPNLPENSFLHFLTSQDYSDEIIYSMVLEIFGLGVDSTAATAVWALSFLVGEQEIQEKLYREINNRTGGQRPVKVVDLKELPYLQAVMKETLRMKPIAPLAVPHVAAKDTTFKGRRIVKGTKVMVNLYAIHHDPNVFPAPYKFMPERFLKDVNSDGRFGDINTMESSLIPFGAGMRICGGVELAKQMVAFALASMVNEFKWDCVSEGKLPDLSEAISFILYMKNPLEAKITPRTKPFRQLEHHHHHH

SEQ ID NO: 22 - DNA, 1482 bp, Papaver somniferum
  misc_feature 1..1482: note = N-terminales Austauschen der Transmembrandomaene (29 Aminosaeuren) mit der Sequenz ALLLAVFL und N-terminales Flanking MG ; C-terminaler His-tag; Codon-optimiert fuer E. coli; Fuer Sequenz-ID Nr. 21 kodierende Sequenz
  source 1..1482: mol_type = genomic DNA
atgggaatggcacttctgctggcagttttccttaagatcagtttctaccagagcgcaaataccaccgaatggccggccggtccgaaaaccctgccgattattggtaatctgcatcagctgggcggcggcgttccgctgcaggttgctctggcaaatctggccaaagtttatggcggtgcctttaccatttggattggtagctgggttccgatgattgttattagtgatattgataacgcccgtgaagttctggttaataagagcgcagattatagcgcacgcgatgtgccggatattctgaaaattattaccgccaatggtaaaaatatcgccgattgcgatagcggcccgttttggcataatctgaaaaaaggcctgcagagctgcattaatccgagtaatgttatgagcctgagtcgcctgcaggaaaaagatatgcagaatctgattaagagcatgcaggaacgcgcaagccagcataatggcattattaagccgctggatcatgcaaaagaagcaagcatgcgtctgctgagtcgtgtgatttttggccatgattttagcaatgaagatctggttattggcgtgaaagatgccctggatgaaatggttcgtattagcggcctggcaagcctggcagatgcattcaaaattgccaaatatctgccgagtcagcgcaaaaatattcgtgatatgtatgccacccgtgatcgtgtgtataatctgattcagccgcatattgttccgaatctgccggaaaatagttttctgcattttctgaccagccaggattatagtgatgaaattatctatagcatggtgctggaaatttttggtctgggtgttgatagtaccgcagcaaccgcagtgtgggccctgagttttctggtgggcgaacaggaaattcaggaaaaactgtatcgcgaaattaataatcgcaccggtggtcagcgtccggttaaagttgtggatctgaaagaactgccgtatctgcaggcagtgatgaaagaaaccctgcgcatgaaaccgattgcaccgctggccgttccgcatgtggccgcaaaagataccacctttaaaggtcgccgcattgttaaaggcaccaaagtgatggttaatctgtatgccattcatcatgatccgaatgtttttccggcaccgtataaattcatgccggaacgttttctgaaagatgtgaatagcgatggccgctttggcgatattaatacaatggaaagcagcctgattccgtttggtgccggtatgcgtatttgtggcggtgtggaactggcaaaacagatggttgcatttgcactggccagtatggttaatgaattcaaatgggattgtgtgagcgaaggcaaactgccggatctgagtgaagccattagctttattctgtatatgaaaaacccgctggaagccaaaattaccccgcgcaccaaaccgtttcgtcagctcgagcaccaccaccaccaccac

SEQ ID NO: 23 - protein, 492 aa, Papaver somniferum
  REGION 1..492: note = N-terminales Austauschen der Transmembrandomaene (29 Aminosaeuren) mit der Sequenz AKKTSS und N-terminales Flanking MG ; C-terminaler His-tag; Codon-optimiert fuer E. coli; Mittels Sequenzierung bestimmte Aminosaeuresequenz
MGMAKKTSSKISFYQSANTTEWPAGPKTLPIIGNLHQLGGGVPLQVALANLAKVYGGAFTIWIGSWVPMIVISDIDNAREVLVNKSADYSARDVPDILKIITANGKNIADCDSGPFWHNLKKGLQSCINPSNVMSLSRLQEKDMQNLIKSMQERASQHNGIIKPLDHAKEASMRLLSRVIFGHDFSNEDLVIGVKDALDEMVRISGLASLADAFKIAKYLPSQRKNIRDMYATRDRVYNLIQPHIVPNLPENSFLHFLTSQDYSDEIIYSMVLEIFGLGVDSTAATAVWALSFLVGEQEIQEKLYREINNRTGGQRPVKVVDLKELPYLQAVMKETLRMKPIAPLAVPHVAAKDTTFKGRRIVKGTKVMVNLYAIHHDPNVFPAPYKFMPERFLKDVNSDGRFGDINTMESSLIPFGAGMRICGGVELAKQMVAFALASMVNEFKWDCVSEGKLPDLSEAISFILYMKNPLEAKITPRTKPFRQLEHHHHHH

SEQ ID NO: 24 - DNA, 1476 bp, Papaver somniferum
  misc_feature 1..1476: note = N-terminales Austauschen der Transmembrandomaene (29 Aminosaeuren) mit der Sequenz AKKTSS und N-terminales Flanking MG ; C-terminaler His-tag; Codon-optimiert fuer E. coli; Fuer Sequenz-ID Nr. 23 kodierende Sequenz
  source 1..1476: mol_type = genomic DNA
atgggaatggcaaagaaaacatcgtctaagatcagtttctaccagagcgcaaataccaccgaatggccggccggtccgaaaaccctgccgattattggtaatctgcatcagctgggcggcggcgttccgctgcaggttgctctggcaaatctggccaaagtttatggcggtgcctttaccatttggattggtagctgggttccgatgattgttattagtgatattgataacgcccgtgaagttctggttaataagagcgcagattatagcgcacgcgatgtgccggatattctgaaaattattaccgccaatggtaaaaatatcgccgattgcgatagcggcccgttttggcataatctgaaaaaaggcctgcagagctgcattaatccgagtaatgttatgagcctgagtcgcctgcaggaaaaagatatgcagaatctgattaagagcatgcaggaacgcgcaagccagcataatggcattattaagccgctggatcatgcaaaagaagcaagcatgcgtctgctgagtcgtgtgatttttggccatgattttagcaatgaagatctggttattggcgtgaaagatgccctggatgaaatggttcgtattagcggcctggcaagcctggcagatgcattcaaaattgccaaatatctgccgagtcagcgcaaaaatattcgtgatatgtatgccacccgtgatcgtgtgtataatctgattcagccgcatattgttccgaatctgccggaaaatagttttctgcattttctgaccagccaggattatagtgatgaaattatctatagcatggtgctggaaatttttggtctgggtgttgatagtaccgcagcaaccgcagtgtgggccctgagttttctggtgggcgaacaggaaattcaggaaaaactgtatcgcgaaattaataatcgcaccggtggtcagcgtccggttaaagttgtggatctgaaagaactgccgtatctgcaggcagtgatgaaagaaaccctgcgcatgaaaccgattgcaccgctggccgttccgcatgtggccgcaaaagataccacctttaaaggtcgccgcattgttaaaggcaccaaagtgatggttaatctgtatgccattcatcatgatccgaatgtttttccggcaccgtataaattcatgccggaacgttttctgaaagatgtgaatagcgatggccgctttggcgatattaatacaatggaaagcagcctgattccgtttggtgccggtatgcgtatttgtggcggtgtggaactggcaaaacagatggttgcatttgcactggccagtatggttaatgaattcaaatgggattgtgtgagcgaaggcaaactgccggatctgagtgaagccattagctttattctgtatatgaaaaacccgctggaagccaaaattaccccgcgcaccaaaccgtttcgtcagctcgagcaccaccaccaccaccac

SEQ ID NO: 25 - protein, 494 aa, Papaver somniferum
  REGION 1..494: note = N-terminales Austauschen der Transmembrandomaene (29 Aminosaeuren) mit der Sequenz KKTSSKGR und N-terminales Flanking MG ; C-terminaler His-tag; Codon-optimiert fuer E. coli; Mittels Sequenzierung bestimmte Aminosaeuresequenz
MGMKKTSSKGRKISFYQSANTTEWPAGPKTLPIIGNLHQLGGGVPLQVALANLAKVYGGAFTIWIGSWVPMIVISDIDNAREVLVNKSADYSARDVPDILKIITANGKNIADCDSGPFWHNLKKGLQSCINPSNVMSLSRLQEKDMQNLIKSMQERASQHNGIIKPLDHAKEASMRLLSRVIFGHDFSNEDLVIGVKDALDEMVRISGLASLADAFKIAKYLPSQRKNIRDMYATRDRVYNLIQPHIVPNLPENSFLHFLTSQDYSDEIIYSMVLEIFGLGVDSTAATAVWALSFLVGEQEIQEKLYREINNRTGGQRPVKVVDLKELPYLQAVMKETLRMKPIAPLAVPHVAAKDTTFKGRRIVKGTKVMVNLYAIHHDPNVFPAPYKFMPERFLKDVNSDGRFGDINTMESSLIPFGAGMRICGGVELAKQMVAFALASMVNEFKWDCVSEGKLPDLSEAISFILYMKNPLEAKITPRTKPFRQLEHHHHHH

SEQ ID NO: 26 - DNA, 1482 bp, Papaver somniferum
  misc_feature 1..1482: note = N-terminales Austauschen der Transmembrandomaene (29 Aminosaeuren) mit der Sequenz KKTSSKGR und N-terminales Flanking MG ; C-terminaler His-tag; Codon-optimiert fuer E. coli; Fuer Sequenz-ID Nr. 25 kodierende Sequenz
  source 1..1482: mol_type = genomic DNA
atgggaatgaagaaaacgagcagtaaaggccgtaagatcagtttctaccagagcgcaaataccaccgaatggccggccggtccgaaaaccctgccgattattggtaatctgcatcagctgggcggcggcgttccgctgcaggttgctctggcaaatctggccaaagtttatggcggtgcctttaccatttggattggtagctgggttccgatgattgttattagtgatattgataacgcccgtgaagttctggttaataagagcgcagattatagcgcacgcgatgtgccggatattctgaaaattattaccgccaatggtaaaaatatcgccgattgcgatagcggcccgttttggcataatctgaaaaaaggcctgcagagctgcattaatccgagtaatgttatgagcctgagtcgcctgcaggaaaaagatatgcagaatctgattaagagcatgcaggaacgcgcaagccagcataatggcattattaagccgctggatcatgcaaaagaagcaagcatgcgtctgctgagtcgtgtgatttttggccatgattttagcaatgaagatctggttattggcgtgaaagatgccctggatgaaatggttcgtattagcggcctggcaagcctggcagatgcattcaaaattgccaaatatctgccgagtcagcgcaaaaatattcgtgatatgtatgccacccgtgatcgtgtgtataatctgattcagccgcatattgttccgaatctgccggaaaatagttttctgcattttctgaccagccaggattatagtgatgaaattatctatagcatggtgctggaaatttttggtctgggtgttgatagtaccgcagcaaccgcagtgtgggccctgagttttctggtgggcgaacaggaaattcaggaaaaactgtatcgcgaaattaataatcgcaccggtggtcagcgtccggttaaagttgtggatctgaaagaactgccgtatctgcaggcagtgatgaaagaaaccctgcgcatgaaaccgattgcaccgctggccgttccgcatgtggccgcaaaagataccacctttaaaggtcgccgcattgttaaaggcaccaaagtgatggttaatctgtatgccattcatcatgatccgaatgtttttccggcaccgtataaattcatgccggaacgttttctgaaagatgtgaatagcgatggccgctttggcgatattaatacaatggaaagcagcctgattccgtttggtgccggtatgcgtatttgtggcggtgtggaactggcaaaacagatggttgcatttgcactggccagtatggttaatgaattcaaatgggattgtgtgagcgaaggcaaactgccggatctgagtgaagccattagctttattctgtatatgaaaaacccgctggaagccaaaattaccccgcgcaccaaaccgtttcgtcagctcgagcaccaccaccaccaccac

SEQ ID NO: 27 - protein, 496 aa, Coptis Japonica
  REGION 1..496: note = N-terminales Flanking MG ; C-terminaler His-tag, Codon-optimiert fuer E. coli; Mittels Sequenzierung bestimmte Aminosaeuresequenz
MGMDLQIALFSLIPVILVFILLLKPKYKNLPPGPHPWPLIGNLPILFTNTEVPLHITLANMARTHGPIMILWLGTQPTVMASTAEAAMEILKTHDRIFSARHIRMSFRLKHHIKYSLVWSDCTDYWKLLRKIVRTEIFSPKMLQAQSHVREQKVAELIDFLRSKEGQVVKISQFVFGTLLNILGNVVFSKDVFVYGDETDKGGIQNLIREMLMIGAEPNVAEFYPSLEELDLQGLKKKCDERFIRVMKMWEGTVKERKANRNEESKDMLDVLLANDFNDAQINALFLETFGPGSETSSATIEWVIAELIKSPKEMAKVRKELNEVVGTSTIKESDLPQLPYLQACIKEAMRLHPAAPFLLPRRAAETCEVMGYTIPKNSQVLVNAYAIGRDPKSWKDPSTFWPERFLESDVDFHGAHYQFIPFGSGRRTCVGMPLATRTIPLIVGSLVHNYDFGLPGGNRPEDLKMNEMLSLTLAIDPSLCVVPKARALEHHHHHH

SEQ ID NO: 28 - DNA, 1488 bp, Coptis Japonica
  misc_feature 1..1488: note = N-terminales Flanking MG ; C-terminaler His-tag, Codon-optimiert fuer E. coli; Fuer Sequenz-ID Nr. 27 kodierende Sequenz
  source 1..1488: mol_type = genomic DNA
atgggaatggatctgcagattgccctgttcagcctgattccggttattctggtgttcattctgctgctgaaaccgaaatataaaaatctgccgccgggcccgcatccgtggcctctgattggtaatctgccgattctgttcaccaataccgaagtgccgctgcatattaccctggcaaatatggcccgtacccacggtccgattatgattctgtggctgggtacccagccgaccgttatggccagtaccgcagaagccgcaatggaaattctgaaaacacatgatcgtatcttcagtgcacgccatattcgtatgagcttccgcctgaaacatcatattaaatatagtctggtgtggagcgattgcaccgattattggaaactgctgcgtaaaattgtgcgcaccgaaatcttcagcccgaaaatgctgcaggcccagagtcatgtgcgcgaacagaaagtggcagaactgattgacttcctgcgtagcaaagaaggtcaggtggttaaaattagtcagttcgtgttcggtaccctgctgaatattctgggtaatgttgtgttcagcaaagatgtgttcgtgtatggtgatgaaaccgataaaggtggtattcagaatctgattcgcgaaatgctgatgattggtgcagaaccgaatgttgcagaattctatccgagcctggaagaactggatctgcagggtctgaaaaaaaaatgtgatgaacgcttcattcgcgttatgaaaatgtgggaaggcaccgtgaaagaacgcaaagcaaatcgcaatgaagaaagtaaagatatgctggatgtgctgctggccaatgacttcaatgatgcacagattaatgccctgttcctggaaaccttcggtccgggtagcgaaaccagcagcgcaaccattgaatgggttattgcagaactgatcaaaagcccgaaagaaatggcaaaagtgcgtaaagaactgaatgaagttgttggcaccagtaccattaaagaaagtgatctgccgcagctgccgtatctgcaggcatgtattaaagaagccatgcgcctgcatccggcagccccgttcctgctgccgcgtagagccgcagaaacctgcgaagtgatgggttataccattccgaaaaatagtcaggtgctggttaatgcatatgcaattggtcgtgatccgaaaagctggaaagatccgagtaccttctggccggaacgcttcctggaaagcgatgttgacttccacggtgcacattatcagttcattccgttcggcagcggtcgccgtacctgcgtgggcatgccgctggcaacccgtaccattccgctgattgtgggtagcctggtgcataattatgacttcggcctgccgggtggtaatcgcccggaagatctgaaaatgaatgaaatgctgagcctgaccctggcaattgatccgagtctgtgtgtggttccgaaagcacgtgccctcgagcaccaccaccaccaccac

SEQ ID NO: 29 - protein, 476 aa, Coptis Japonica
  REGION 1..476: note = N-terminales Entfernen der Transmembrandomaene (21 Aminosaeuren) und N-terminales Flanking MG ; C-terminaler His-tag; Codon-optimiert fuer E. coli; Mittels Sequenzierung bestimmte Aminosaeuresequenz
MGMKPKYKNLPPGPHPWPLIGNLPILFTNTEVPLHITLANMARTHGPIMILWLGTQPTVMASTAEAAMEILKTHDRIFSARHIRMSFRLKHHIKYSLVWSDCTDYWKLLRKIVRTEIFSPKMLQAQSHVREQKVAELIDFLRSKEGQVVKISQFVFGTLLNILGNVVFSKDVFVYGDETDKGGIQNLIREMLMIGAEPNVAEFYPSLEELDLQGLKKKCDERFIRVMKMWEGTVKERKANRNEESKDMLDVLLANDFNDAQINALFLETFGPGSETSSATIEWVIAELIKSPKEMAKVRKELNEVVGTSTIKESDLPQLPYLQACIKEAMRLHPAAPFLLPRRAAETCEVMGYTIPKNSQVLVNAYAIGRDPKSWKDPSTFWPERFLESDVDFHGAHYQFIPFGSGRRTCVGMPLATRTIPLIVGSLVHNYDFGLPGGNRPEDLKMNEMLSLTLAIDPSLCVVPKARALEHHHHHH

SEQ ID NO: 30 - DNA, 1428 bp, Coptis Japonica
  source 1..1428: mol_type = genomic DNA
  misc_feature 1..1428: note = N-terminales Entfernen der Transmembrandomaene (21 Aminosaeuren) und N-terminales Flanking MG; C-terminaler His-tag; Codon-optimiert fuer E. coli; Fuer Sequenz-ID Nr. 29 kodierende Sequenz
atgggaatgaaaccgaaatataaaaatctgccgccgggcccgcatccgtggcctctgattggtaatctgccgattctgttcaccaataccgaagtgccgctgcatattaccctggcaaatatggcccgtacccacggtccgattatgattctgtggctgggtacccagccgaccgttatggccagtaccgcagaagccgcaatggaaattctgaaaacacatgatcgtatcttcagtgcacgccatattcgtatgagcttccgcctgaaacatcatattaaatatagtctggtgtggagcgattgcaccgattattggaaactgctgcgtaaaattgtgcgcaccgaaatcttcagcccgaaaatgctgcaggcccagagtcatgtgcgcgaacagaaagtggcagaactgattgacttcctgcgtagcaaagaaggtcaggtggttaaaattagtcagttcgtgttcggtaccctgctgaatattctgggtaatgttgtgttcagcaaagatgtgttcgtgtatggtgatgaaaccgataaaggtggtattcagaatctgattcgcgaaatgctgatgattggtgcagaaccgaatgttgcagaattctatccgagcctggaagaactggatctgcagggtctgaaaaaaaaatgtgatgaacgcttcattcgcgttatgaaaatgtgggaaggcaccgtgaaagaacgcaaagcaaatcgcaatgaagaaagtaaagatatgctggatgtgctgctggccaatgacttcaatgatgcacagattaatgccctgttcctggaaaccttcggtccgggtagcgaaaccagcagcgcaaccattgaatgggttattgcagaactgatcaaaagcccgaaagaaatggcaaaagtgcgtaaagaactgaatgaagttgttggcaccagtaccattaaagaaagtgatctgccgcagctgccgtatctgcaggcatgtattaaagaagccatgcgcctgcatccggcagccccgttcctgctgccgcgtagagccgcagaaacctgcgaagtgatgggttataccattccgaaaaatagtcaggtgctggttaatgcatatgcaattggtcgtgatccgaaaagctggaaagatccgagtaccttctggccggaacgcttcctggaaagcgatgttgacttccacggtgcacattatcagttcattccgttcggcagcggtcgccgtacctgcgtgggcatgccgctggcaacccgtaccattccgctgattgtgggtagcctggtgcataattatgacttcggcctgccgggtggtaatcgcccggaagatctgaaaatgaatgaaatgctgagcctgaccctggcaattgatccgagtctgtgtgtggttccgaaagcacgtgccctcgagcaccaccaccaccaccac